European Patent Application EP 4 610 354 A1, published September 3, 2025. Title: ゲノム編集方法およびゲノム編集用組成物. Applicant: 株式会社インプランタイノベーションズ. Application JP. The sequence listing filed with the application follows.

SEQUENCE LISTING (44 sequences)

SEQ ID NO: 1-3 - skipped (3 entries)

SEQ ID NO: 4 - protein, 3177 aa, Abyssicoccus albus
METLYSHISSERGLYGLNTYRILELEUGLYLEUASPILEGLYILEALASERVALGLYTYRGLYLEUILEASNASNASPTHRLYSGLUILEILEASPALAGLYVALARGLEUPHEPROGLUGLYLYSSERASPGLUASNASPGLYARGARGSERLYSARGGLYSERARGARGLEULEUARGARGARGLYSHISARGILEALAASNVALLYSSERLEULEUALAGLUTYRGLYILESERILEGLUASNASNSERASNMETASNPROTYRGLUILEARGVALLYSGLYLEUSERGLULYSLEUSERASPGLUGLULEUALAALAALALEUILEHISLEUSERLYSARGARGGLYILEHISASNVALASPVALTHRASPASPSERGLUGLUSERSERGLULEUSERTHRLYSASPGLNILEASNARGASNALALYSLEULEUTHRASPLYSHISVALALAGLULEUGLNLEUGLUARGLEUASNASNGLUGLYSERVALARGGLYHISSERASNARGPHELYSTHRASNASPTYRILELYSGLUALAGLUALALEULEUASPLYSGLNILEGLUTYRASNGLNLYSILEASPGLYGLUPHELYSARGLYSTYRILEHISLEUILEASNARGARGARGALATYRTYRGLUGLYPROGLYGLUGLYSERPROPHEGLYTRPASNALAASPILELYSLYSTRPTYRGLUTHRLEUMETGLYLYSCYSTHRTYRTYRPROGLUGLULEUARGSERVALARGTYRALATYRSERALASERLEUPHEASNVALLEUASNASPLEUASNASNLEUVALILEMETARGASPGLUASNASPLYSLEUTHRLYSASPGLULYSGLUHISLEUILEASNASNLEUPHELYSLYSGLNLYSSERALAPROTHRLEUASNLYSILEALALYSGLULEUGLYVALLYSGLUGLUASPILELYSGLYTYRARGVALASPLYSLYSASPLYSPROGLUPHESERTHRILELYSILETYRHISASPILELYSGLYILETHRASNASNPROGLUILELEUGLUASNPROASPVALLEUASPLYSILEALAGLUILELEUTHRILETRPGLNASNGLULYSHISILELEUGLUGLULEUGLULYSLEUGLNLEUASNLEUASNGLUGLNGLUARGVALLYSVALALAASNLEUTHRGLYTYRTHRGLYTHRHISSERLEUSERLEULYSLEUILELYSGLNLEUASNSERGLULEUTRPGLUSERTHRLEUASNHISMETGLYILEILESERASNMETASNLEUARGPROLYSLYSMETGLUPHELYSGLYLEUASPLYSILEPROVALASPPHEVALASPGLUTRPILELEUSERPROALAVALLYSARGSERLEUILEGLNSERILELYSVALVALASNGLUILEILELYSVALTYRGLYGLUPROLYSASPILEILEILEGLULEUALAARGGLUSERASNSERASPASPLYSLYSLYSPHELEUGLNLYSLEUGLNLYSASPSERGLNLYSILEASNGLUGLNVALARGALALYSILESERGLUILEASNGLYLYSASPASNPHESERSERSERLEUPHEGLULYSVALLYSLEUTRPHISLEUGLNASPGLYLEUCYSMETTYRSERTHRGLUSERILELYSILEASPASPLEUILEGLNASNPROASNALATYRGLUVALASPHISILEILEPROARGSERVALSERPHEASPASPSERLEUASNASNLYSVALLEUVALLYSLEUGLUGLUASNGLNLYSLYSSERASNMETTHRPROTYRGLNTYRLEUSERSERGLYGLNGLYSERILESERTYRGLULYSPHELYSALAASNVALLEUTHRLEUALALYSASPGLYLYSARGILESERLYSLYSLYSARGGLYTYRLEULEUGLUGLUARGASPILEASNLYSPHEGLUVALGLNLYSGLUPHEILEASNARGASNLEUVALASPTHRARGTYRTHRTHRARGGLULEUMETASNLEULEULYSLEUTYRPHELYSASPASNGLUMETLYSTHRLYSVALLYSALAILEASNGLYGLYPHETHRHISALALEUARGLYSILETRPGLYPHEASNLYSASPARGSERGLUASPTYRLYSHISHISALAGLUASPALALEUILEILEALAMETALAASPTYRILEPHEALAASNLYSASPILEPHELYSASNGLNASNILELEUMETARGASPASNGLNALAILEASPLEUGLUTHRGLYGLUILELEUSERGLULYSASPPHEVALASPARGPHEPHEGLUASPGLUVALPHESERASNILEARGALAILELYSASNPHEASPARGTYRLYSTYRSERLYSARGVALASPLYSLYSPROASNARGGLNLEUMETASNGLUTHRILETYRSERSERARGTHRPHEASPASPGLYGLUTYRILEILEGLYLYSLEULYSASNLEUTYRASPPROLYSASNLYSASPVALLYSLYSLYSILEASNLYSASNPROGLNALAPHELEUMETTYRHISHISASPPROGLNTHRPHEGLULYSLEUGLNTHRILELEUASPGLNTYRSERASPALAASPASNPROLEUALALYSTYRTYRGLUGLUTHRGLYGLUPHELEULYSLYSTYRSERLYSGLUGLYASNGLYPROVALVALLYSSERLEULYSTYRLYSTYRARGLYSLEUGLYALAHISHISASPILETHRASPLYSTYRGLNARGSERARGASNLYSVALPHETHRLEUSERLEULYSPROPHEARGILEASPILETYRLYSASPGLYGLYLYSTYRLYSPHEVALASNILEASNTYRILEASPVALLYSASPVALGLYSERGLUTYRASNVALASPGLUASNSERTYRASNGLULYSLYSASNARGLYSASNILETHRGLUGLNALAGLUPHEILEGLYSERPHEPHELYSTYRASPLEUILELYSILEASPASPGLNLEUTYRSERLEUILESERILEHISSERGLUSERSERASNLYSLEUGLUVALASPLEUVALASNLYSSERTYRLYSGLUTYRALAGLULYSASNLYSLEUASNLYSGLNLYSTYRILESERILEGLYSERLYSASNASNILETHRLYSTYRTHRTHRASPILELEUGLYASNLEUTYRPROVALTYRASNGLULYSLEULYSMETLYSPHEPROLYSTYRLYSGLYASNGLU

SEQ ID NO: 5 - DNA, 3180 bp, Abyssicoccus albus
  source 1..3180: mol_type = other DNA
ttgaaacatagtggacaatacatattagggttagatattggtatcgcttcagtaggttacgggttaattaataatgatactaaagaaattattgatgctggagttcgtttgtttccagaaggtaaaagtgatgaaaatgatgggagaagatcaaagagaggttctagacgtttactcagaaggcgtaaacatagaattgcaaatgtgaagtcgttattagcggaatatggtatttctatagagaataatagtaatatgaatccttatgaaattcgagttaaaggattatcagaaaaacttagtgatgaagaattagcagcagctttaattcatctatcaaaaagaagaggaatacataatgtcgatgttacagatgattctgaagaaagttcagaactttcgacaaaagatcaaattaatagaaatgccaaattattaactgataagcatgtagcggaattacagttagaaagattaaataatgaaggatcagttagagggcactcaaacagatttaaaaccaatgattatataaaagaagcggaagctttattagataaacaaattgagtataaccaaaagatagatggtgaatttaagagaaaatatattcatctaataaatagaagaagagcatactatgaaggacctggtgaaggaagtccatttggatggaatgctgatattaagaaatggtatgaaactttaatgggtaaatgtacatattatcctgaagagttaagatcggtaagatatgcttattctgcttctttattcaatgtcctgaacgacctaaataatttagtcattatgagagatgaaaatgataagttaacaaaagatgaaaaagaacatttaattaataatttgtttaaaaagcaaaaatcagcacctaccttaaataagattgctaaagagcttggggtaaaagaagaagatataaaaggatatcgagttgataaaaaggataaacctgaattttcaacgattaaaatttatcatgatattaaaggaattacgaataatccagagatactagaaaatcctgatgtattagataagattgccgagattttaacgatttggcaaaatgaaaaacacatcttagaagaattggaaaagttacaacttaatttaaacgagcaagaaagagtcaaagtggcaaatcttactggatatacaggtacgcactcattatctttaaagcttataaaacaattgaattcagaactatgggagtccaccctaaatcatatgggtattatatcgaatatgaatttaaggccaaagaaaatggaatttaaggggttagataaaattccggttgactttgtagatgagtggatcttatcaccagcagtaaaaagaagcttaattcaatctattaaagtcgtaaatgaaattataaaagtatatggtgagcctaaagatatcatcattgaattggcaagagagtcgaatagtgatgataagaaaaaatttttacaaaagttacagaaagacagtcaaaaaataaatgaacaagttagagctaagatttctgagattaatgggaaagataatttttcaagtagtctctttgagaaagtgaaattatggcatctacaagatggtttatgtatgtattctactgaatcgataaaaattgatgatttaatacagaacccaaatgcatatgaagtagaccatatcattccaagatcagtgtcttttgatgattctcttaataataaagtattagttaaattagaagagaatcaaaagaaatcaaatatgacaccatatcaatatttgagttcaggacaagggtcaatcagttatgaaaaatttaaagcgaatgtcctcactttagcgaaagatggtaaaagaatctctaaaaagaaaagaggatatctcttagaagaacgtgacataaacaaattcgaagttcaaaaagaattcattaatagaaatctggttgacactaggtatacgacaagagagctaatgaatttattaaaattgtactttaaagataatgaaatgaagacaaaagttaaagcgattaatggtgggttcactcatgcactacgtaaaatatgggggttcaataaagatcgtagtgaagattataaacatcatgctgaagatgctttaataatagctatggcagattatatttttgcaaataaagatatctttaaaaaccaaaatattttaatgcgagacaaccaagcgatagatctagagactggtgaaattttatctgagaaagactttgtagatagattttttgaagatgaagtgtttagtaacattagagcaattaaaaattttgatcgttataaatattctaagcgtgttgataaaaaaccgaacaggcaattaatgaatgaaacaatttattcatcaagaacatttgatgatggtgaatacattatcgggaaacttaaaaatttatatgatccaaaaaataaggatgttaaaaagaaaattaataaaaatccacaggcatttttaatgtatcatcatgacccacaaacatttgaaaaattacaaacaattttagatcaatatagtgatgctgataacccactcgctaagtactatgaagaaactggtgaattcttgaagaagtatagtaaagaaggtaacggaccagttgtgaagagtctgaaatataaatatagaaaattaggagcacatcatgatattactgataaatatcaaagatcacgtaacaaagtatttacattaagtttaaagcctttccgtattgatatatataaagacggtgggaagtataagtttgtaaatattaattatattgatgtgaaagatgtaggatctgaatataatgtcgatgagaatagttacaatgaaaaaaagaatcgaaagaatatcactgagcaagcagaatttattggatcattttttaaatatgacttaattaagattgatgatcaactttatagccttattagtattcatagtgaaagttccaataagctagaggttgatttagtgaataaaagctataaagaatatgcagaaaaaaacaaactaaataaacaaaagtatataagtataggttctaaaaataatatcactaagtatacaactgatatactaggcaatttatacccagtttataatgagaaattaaaaatgaaattcccaaaatacaaaggtaatgagtaa

SEQ ID NO: 6 - DNA, 3177 bp, synthetic construct
  source 1..3177: mol_type = other DNA
atgaagcactctgggcaatatattctgggtcttgacatcggtatcgcttccgtaggctacggattaatcaataacgataccaaggaaattatcgacgccggggttcgtctgtttccggaaggcaaaagcgatgagaatgatgggcgtcgtagcaagcgtggcagtcgccgtcttttgcgtcgtcgcaaacaccgtattgcaaatgtgaaatctttgcttgctgaatatggcattagcattgagaacaactcaaacatgaatccttatgaaatccgcgtcaaaggactttccgaaaagttgtcagatgaggagcttgccgctgcgttgattcacttgtctaagcgtcgcggcatccataacgtggatgtcactgatgacagcgaagaatcatcagagttaagtacaaaggatcaaattaaccgcaatgcaaaattactgacggacaagcatgtagcggaattgcaactggagcgcctgaacaacgaagggtcggtacgcggccattctaaccgctttaaaacgaatgattatattaaagaagccgaagcacttttggataagcaaattgagtacaaccagaaaatcgatggggaatttaaacgcaaatatatccacttaatcaatcgtcgccgtgcctactatgaggggccaggggagggtagcccgtttggctggaatgcggatattaagaaatggtatgaaaccttaatgggcaaatgcacttattatccagaggaattacgctcggtacgctacgcatactcggcttctcttttcaacgttttaaacgatctgaataacttggtgatcatgcgtgacgagaatgacaaattgacgaaagacgagaaggaacatttaatcaataatctgttcaaaaaacaaaagtcggctccgactttaaataagattgcaaaagagctgggggtaaaagaggaagacatcaaaggatatcgtgtcgacaaaaaggacaagccggagttttccacaattaaaatttaccatgatatcaaaggtattactaacaatccagagattttagagaatccagatgtacttgataagattgccgagattttgactatttggcagaacgagaagcatattctggaagaactggagaaattgcagcttaacttgaatgagcaagaacgtgtcaaagtagcgaatcttaccgggtacactggcacccactcgctttctctgaaattaatcaagcaactgaactcagagttgtgggagtccactttgaatcatatgggaatcattagtaacatgaacttgcgtccgaaaaagatggaattcaagggattagataagatccctgtcgacttcgttgatgagtggattttaagtcctgccgtgaagcgtagtttaatccaatcgattaaagtggttaatgaaattattaaagtttacggagagccgaaagatatcatcatcgaacttgctcgtgagtcgaacagcgatgacaaaaagaaatttttgcagaaattgcaaaaagattcccaaaagattaacgagcaagtgcgcgccaagatctccgaaattaacggaaaagataattttagctcgagcttatttgaaaaagtgaagctttggcatcttcaggatgggttatgtatgtacagcactgagagcattaaaattgatgaccttattcagaatccaaatgcctacgaggtagatcatatcatcccacgttcggtatcttttgatgatagtcttaacaacaaggtccttgtaaagttagaagaaaaccagaagaagtcgaatatgaccccataccaatatctgagctccggtcagggatcgatctcttacgagaagtttaaggccaatgtacttaccctggctaaggatggcaagcgcatcagcaagaaaaagcgtgggtacctgttagaggagcgtgatatcaataaattcgaggtgcaaaaggaatttattaatcgtaatttggtggacactcgctacactacccgcgagctgatgaatttattaaagctttatttcaaagataacgagatgaagacaaaggtgaaggccattaatgggggctttacacacgcgctgcgcaaaatctgggggttcaacaaagatcgctcagaagactataagcatcatgcagaggatgcattgatcattgctatggccgattacatttttgcgaataaagacatcttcaaaaatcagaacattttgatgcgcgataaccaagccatcgatttagaaaccggagagatcttaagtgaaaaagatttcgtggaccgcttctttgaggacgaggtgttcagtaatattcgtgcaattaagaacttcgaccgttataaatatagtaagcgtgtagataaaaaacctaaccgtcaacttatgaacgagaccatttactcttcacgcacgtttgacgatggcgagtatattattggcaaacttaaaaacttgtacgatccaaagaacaaagacgtcaaaaagaaaattaacaagaacccccaggcattcttaatgtatcaccatgacccgcagacatttgagaaattacagacgattttagatcagtattcggacgcagataaccccttagccaaatactatgaggaaacaggagaatttttgaagaaatatagcaaggaagggaatggaccggtagttaaaagtttaaagtataagtaccgtaaactgggtgctcaccatgatatcaccgacaagtaccagcgttctcgtaataaagtgtttacgctttcgctgaagcccttccgtattgacatctataaggacggcggtaagtacaaatttgtaaacattaactacatcgatgttaaggatgtaggctcagaatataacgtagatgaaaactcatacaacgaaaagaaaaaccgcaagaacattaccgagcaagcagaatttattggttctttttttaagtatgacttaatcaaaattgacgatcagttatatagcttaatcagcattcattcagagtcttcaaacaagttagaggtagacctggtaaataaatcttacaaggaatacgcagagaaaaacaagctgaacaagcaaaagtatatctcaatcggctcaaaaaataacattacaaaatacacgaccgacattttagggaacctgtatcctgtttacaatgaaaagctgaaaatgaaattcccgaagtataagggcaatgag

SEQ ID NO: 7 - DNA, 3177 bp, synthetic construct
  source 1..3177: mol_type = other DNA
atgaagcactctgggcaatatatcttgggattggatataggcatagcaagtgtaggttatggcttgatcaacaatgacacgaaagagattatcgacgcaggggtgcgactctttccggaaggtaagagcgatgaaaacgatggacgccgcagcaaacgcggctcacgaagattgttgagacgccgcaagcacagaatcgcgaacgtaaaatccctgctggccgaatatggaatttcaattgaaaacaactctaacatgaatccatacgagattcgcgtaaaaggcctgtccgaaaaattgtctgatgaggaactcgcggcggcactcatacatcttagcaagcggagggggattcataatgtcgacgtcacggacgattccgaggaatcttctgaacttagcaccaaagaccagatcaatcgcaacgccaaattgcttactgataagcatgttgcagagcttcagctggagcgcctcaataatgaagggagtgtccgaggccatagcaataggttcaagacaaacgactacattaaggaggcggaagcgctgcttgataagcaaatcgaatacaaccagaagatcgacggagagttcaaacgaaaatatattcatttgatcaatcgacgccgagcgtactatgaaggtccgggggaagggtctccctttggctggaatgccgacatcaaaaagtggtatgaaactctcatgggcaaatgcacttattatcccgaggagcttagatctgtgaggtatgcttatagcgcaagtctcttcaatgtccttaacgatcttaacaaccttgtgattatgcgggatgaaaacgataagttgaccaaggatgaaaaagagcatctcattaacaaccttttcaaaaagcaaaaatcagcccccacactgaacaagatagcgaaggaacttggtgtaaaggaggaggacatcaaagggtacagggtggataaaaaagataagcccgaattcagtacgattaaaatctaccacgatataaaaggtataacgaacaatcctgaaattctcgaaaaccccgacgtccttgataaaattgctgaaatattgacaatctggcagaacgaaaagcatatactggaggaactcgaaaagctgcaattgaatttgaatgagcaggaacgggtgaaagtcgccaatttgaccggctacacagggactcatagtctgagcctcaaacttatcaaacagctcaatagtgaattgtgggagagtacccttaatcacatgggcatcataagcaatatgaatctgagaccaaagaagatggagtttaaaggactcgataaaatacctgttgacttcgtagacgagtggatcttgtcacccgcagtaaagcgcagtctgatccaaagcatcaaggtcgtcaacgaaattattaaagtttacggggagccgaaggacataataatagaattggcgcgagaaagcaactcagatgataagaagaaattcttgcagaaacttcaaaaagattcacaaaagatcaacgaacaggtacgggctaaaatttctgagattaacggaaaagacaattttagttcttctctcttcgagaaagttaaactctggcatctgcaagatgggttgtgcatgtattcaaccgaatctataaagatagacgatctgatccagaatccgaatgcttatgaagtagaccacatcattccgcgctctgtctcttttgatgattcccttaacaacaaagtacttgttaagcttgaggaaaatcagaaaaagtccaacatgacgccgtaccagtacctctcttcaggtcagggtagcatatcctatgagaaatttaaagcgaatgtactgacgctcgccaaagatgggaagaggatctctaagaaaaaacgaggatatttgctcgaagagagggacattaataagttcgaggtgcagaaagagtttataaatcggaatctcgtagatacccgatatacgactcgggaattgatgaaccttcttaagctctattttaaggataacgagatgaaaacgaaagtcaaggctataaacggcgggttcactcatgccctgaggaaaatatgggggtttaataaagaccgctcagaagactataagcaccatgcggaggacgcgctgattattgcgatggcagattatattttcgcaaacaaagacatatttaagaaccaaaatatcctcatgcgggataatcaggccattgatcttgaaactggagagatcctcagtgagaaggatttcgtggatagattcttcgaggacgaggtcttcagcaatatacgcgcaataaagaatttcgatagatataagtattctaagagagtagataaaaagccgaatcgacagctgatgaatgagacgatatactcctcacgcacgtttgatgacggagagtacataatcggcaagctcaagaatctgtacgaccctaaaaataaggatgtaaagaaaaaaataaacaagaatccacaagcattcttgatgtatcaccacgacccccaaacgtttgagaaactgcaaacaatattggatcagtattccgatgcagacaatccgttggcgaaatactacgaggaaacgggcgagtttcttaagaaatattctaaggagggcaacggacccgtagtcaagtcactgaaatataaatacaggaaactcggggctcaccatgacataacggacaaataccagcgatcacgaaacaaagtattcacactctctttgaagcctttccgcatcgatatctacaaggacggtgggaaatacaagtttgtgaacattaactacatagacgtcaaggacgtaggcagtgaatataacgtagatgagaattcttacaatgaaaagaagaatcgaaaaaacataactgaacaggctgagttcattggatccttctttaaatatgaccttattaaaattgatgatcaactgtacagcttgatatctatacatagtgagtccagtaacaagttggaggtggatctggttaataaaagttataaagaatatgccgaaaagaataagctcaataagcagaagtatatctcaattgggtccaaaaacaatattacgaagtacactacagacatcctcggcaatctctatcccgtatataatgaaaaactgaaaatgaaatttcccaagtataaaggtaacgag

SEQ ID NO: 8 - DNA, 3177 bp, synthetic construct
  source 1..3177: mol_type = other DNA
atgaagcatagcggccaatatatactcgggctcgatattggtatagctagcgtgggctacggactcataaacaatgacacgaaagaaatcatcgatgcaggtgtcaggttatttccggaaggtaaatctgatgaaaacgatggtaggaggagcaagagaggatcaagacgtttgctaaggaggaggaaacacagaattgctaacgtcaagagtttactggccgagtatggtatctccattgaaaataattccaacatgaatccttacgagataagggtgaagggccttagcgaaaaactgtccgacgaggaactagctgctgccttaattcacctgagtaagagacgaggcatacataacgttgacgtaactgatgattcagaggagagttcagaactaagcaccaaagaccaaataaatagaaatgccaaattactgacggacaagcatgttgctgaactgcagctggagaggctaaacaatgaaggatctgtccgaggacacagcaatcgattcaagaccaacgactatataaaagaagcagaagcactcctcgataaacagattgagtacaaccaaaagatcgacggtgagtttaaacgtaagtatatacatttgattaacagacgacgtgcgtactatgaaggccctggggagggtagcccgttcggatggaatgcagacattaagaagtggtacgagacccttatggggaagtgtacatattacccagaggaactacgatctgtccgttacgcttactctgcttccctatttaacgtactcaatgatctcaataatctggtaattatgagggatgaaaatgataaattgacaaaggacgagaaagagcatctaatcaacaacctctttaagaagcagaaaagcgctccgacgctaaacaaaattgcgaaggaactcggggtaaaagaagaagacataaagggataccgagtcgacaaaaaagataagccggaattttccacgattaagatctatcatgacataaaggggatcacaaataacccggaaattcttgagaatccggatgttttggacaagattgctgagatattgacgatttggcagaacgaaaaacacattcttgaagagttggaaaagctccaactgaatcttaacgaacaggaacgtgtaaaagtggcaaatctaacagggtatacaggaacacacagcctatcattgaaattgatcaagcagctgaactccgaactttgggagtccaccctcaaccacatgggtattataagtaatatgaatctgagacctaaaaagatggaattcaagggtctcgacaagatacctgtagactttgtcgacgagtggatcttatccccagctgtgaagcgttcactgatccaatctataaaggtagtaaatgaaataatcaaggtttatggtgagcctaaagatattatcatagaattggcacgtgaaagcaacagcgacgacaagaagaaattcctgcaaaagctacagaaagactctcaaaagatcaacgagcaagttcgtgcaaagatttccgaaataaacggcaaagacaatttttctagttctttatttgagaaagttaagctctggcaccttcaagatggactgtgcatgtactccactgaatctattaagatagacgacctcattcagaacccgaatgcctatgaggttgatcatattatcccccgttcagtctctttcgacgattccctaaataataaagttcttgtgaagctggaggaaaaccaaaaaaagagtaatatgacgccctaccagtatttaagcagtggtcagggctccatttcttatgaaaagtttaaggctaacgttttaactttggcaaaagacgggaagcgaattagcaaaaaaaagagaggatatctacttgaagagcgtgatatcaacaagtttgaggtgcaaaaggaattcataaataggaatcttgtagatacgaggtacaccacccgtgaactcatgaatcttctcaaactttattttaaagacaatgagatgaaaaccaaagtaaaagcgattaacggcgggttcactcacgccctccgtaaaatctgggggtttaacaaggatcgttctgaggattataagcaccacgctgaagatgccttgataatagcgatggccgattacatttttgctaacaaggatatctttaagaaccaaaatattctcatgcgagataaccaagcaatagatctggagacaggcgaaatcctgagtgaaaaggatttcgttgatagattttttgaggatgaagtcttttctaacatccgagcgataaaaaactttgaccgttacaagtattctaagagagtagataaaaaaccgaacaggcaactgatgaatgagaccatctactcctcccgaacatttgacgacggagaatacattatcggtaagctaaaaaacctatacgatcccaagaataaggatgttaagaaaaagatcaacaaaaatccccaagcctttctaatgtaccaccatgaccctcaaacattcgaaaagcttcaaacgatacttgaccagtatagtgatgcagataaccctttagcgaagtactacgaagaaacaggagagtttctcaaaaaatatagcaaagaaggaaacggccctgtagtaaagtctctaaagtataagtataggaaacttggcgctcatcatgatattactgacaagtatcagcgtagccgaaacaaagtctttacgctttctctcaaaccgttcaggattgacatttacaaagacggtgggaaatataaatttgtcaatataaattatatagacgtcaaggacgtcggtagcgaatataacgtagacgaaaatagctacaacgaaaagaagaatagaaagaatattaccgagcaagccgagtttataggttctttcttcaagtatgatctgataaagattgacgaccaactttatagtctaattagtatacactcagagtcaagcaacaaattagaggtggatttagttaataagtcctacaaagaatatgcagagaagaacaaattaaataaacaaaaatacatcagcataggctccaaaaacaatataacaaagtatactacggacatcctgggcaacttataccccgtttataacgaaaagctcaagatgaagtttccgaagtacaaaggaaatgag

SEQ ID NO: 9 - DNA, 66 bp, synthetic construct
  source 1..66: mol_type = other DNA
tcctccagagactttccgcttcttctttggggctttatgattcatatgtatatctccttcttaaag

SEQ ID NO: 10 - DNA, 78 bp, synthetic construct
  source 1..78: mol_type = other DNA
tctggcggctcaaaaagaaccgccgacggcagcgaattcgagcccaagaagaagaggaaagtcctcgagcaccaccac

SEQ ID NO: 11 - DNA, 18 bp, synthetic construct
  source 1..18: mol_type = other DNA
cggaaagtctctggagga

SEQ ID NO: 12 - DNA, 18 bp, synthetic construct
  source 1..18: mol_type = other DNA
gcgctaagaacgagcgcg

SEQ ID NO: 13 - DNA, 27 bp, synthetic construct
  source 1..27: mol_type = other DNA
gatcgttggtctttgctcctgcagagg

SEQ ID NO: 14 - DNA, 27 bp, synthetic construct
  source 1..27: mol_type = other DNA
aattcctctgcaggagcaaagaccaac

SEQ ID NO: 15 - DNA, 41 bp, synthetic construct
  source 1..41: mol_type = other DNA
acatctgacgctgccgacgacaagcttggcactggccgtcg

SEQ ID NO: 16 - DNA, 22 bp, synthetic construct
  source 1..22: mol_type = other DNA
ccggaagcataaagtgtaaagc

SEQ ID NO: 17 - DNA, 62 bp, synthetic construct
  source 1..62: mol_type = other DNA
cttgtcgtcggcagcgtcagatgtgtataagagacagcatgcctgcaggtcgactcgagagg

SEQ ID NO: 18 - DNA, 72 bp, synthetic construct
  source 1..72: mol_type = other DNA
acactttatgcttccgggtctcgtgggctcggagatgtgtataagagacagctcgtatgttgtgtggaattg

SEQ ID NO: 19 - DNA, 17 bp, synthetic construct
  source 1..17: mol_type = other DNA
ggtctttgctcctgcag

SEQ ID NO: 20 - DNA, 48 bp, synthetic construct
  source 1..48: mol_type = other DNA
agctatgaccatgattacgaattcnnnnnnnctgcaggagcaaagacc

SEQ ID NO: 21 - DNA, 17 bp, synthetic construct
  source 1..17: mol_type = other DNA
ctgcaggagcaaagacc

SEQ ID NO: 22 - DNA, 24 bp, synthetic construct
  source 1..24: mol_type = other DNA
gtaatcatggtcatagctgtttcc

SEQ ID NO: 23 - RNA, 104 nt, synthetic construct
  source 1..104: mol_type = other RNA
gttttagtactctgcgaaatttagtgaaaactagatttcgcagaatctattaaaacaaggctttatgccgtatttaactccatcctatgggtggggtatttttt

SEQ ID NO: 24 - DNA, 31 bp, synthetic construct
  source 1..31: mol_type = other DNA
gcgatcggtgcgggcctcttcgctattacgc

SEQ ID NO: 25 - DNA, 29 bp, synthetic construct
  source 1..29: mol_type = other DNA
attaggcaccccaggctttacactttatg

SEQ ID NO: 26 - DNA, 66 bp, synthetic construct
  source 1..66: mol_type = other DNA
cggataacaatttcacacaggaaacagctatgaccatgattacgaattctgcgttactgcaggagc

SEQ ID NO: 27 - DNA, 31 bp, synthetic construct; identical to SEQ ID NO: 24
  source 1..31: mol_type = other DNA

SEQ ID NO: 28 - DNA, 66 bp, synthetic construct
  source 1..66: mol_type = other DNA
cggataacaatttcacacaggaaacagctatgaccatgattacgaattctttcccactgcaggagc

SEQ ID NO: 29 - RNA, 135 nt, synthetic construct
  source 1..135: mol_type = other RNA
gtagcgagtaatcgtgaagtagagaaacagggttttagtactctgcgaaatttagtgaaaactagatttcgcagaatctattaaaacaaggctttatgccgtatttaactccatcctatgggtggggtatttttt

SEQ ID NO: 30 - RNA, 102 nt, synthetic construct
  source 1..102: mol_type = other RNA
ggacttttgccagccatggtgttttagagctagaaatagcaagttaaaataaggctagtccgttatcaacttgaaaaagtggcaccgagtcggtgctttttt

SEQ ID NO: 31 - DNA, 61 bp, synthetic construct
  source 1..61: mol_type = other DNA
tcgtcggcagcgtcagatgtgtataagagacagggaaaagaatcatatggtcatcaattcg

SEQ ID NO: 32 - DNA, 62 bp, synthetic construct
  source 1..62: mol_type = other DNA
gtctcgtgggctcggagatgtgtataagagacagcggacttgaattaaaggggctatagtag

SEQ ID NO: 33 - DNA, 60 bp, synthetic construct
  source 1..60: mol_type = other DNA
tcgtcggcagcgtcagatgtgtataagagacaggcaaataattaaagttgttgctgttgg

SEQ ID NO: 34 - DNA, 55 bp, synthetic construct
  source 1..55: mol_type = other DNA
gtctcgtgggctcggagatgtgtataagagacagtagcctacttgcctgcttttc

SEQ ID NO: 35 - protein, 17 aa, synthetic construct
MAPKKKRKVGIHGVPAA

SEQ ID NO: 36 - protein, 16 aa, synthetic construct
KRPAATKKAGQAKKKK

SEQ ID NO: 37 - RNA, 493 nt, synthetic construct
  source 1..493: mol_type = other RNA
ctttttttcttcttcttcgttcatacagtttctttttgtttatcagcttacattttcttgaaccgtagctttcgttttcttctttttaactttccattcggagtttttgtatcttgtttcatagtttgtcccaggattagaatgattaggcatcgaaccttcaagaatttgattgaataaaacatcttcattcttaagatatgaagataatcttcaaaaggcccctgggaatctgaaagaagagaagcaggcccatttatatgggaaagaacaatagtatttcttatataggcccatttaagttgaaaacaatcttcaaaagtcccacatcgcttagataagaaaacgaagctgagtttatatacagctagagtcgaagtagtgattgggagaccgagagagggtctcagttttagagctagaaatagcaagttaaaataaggctagtccgttatcaacttgaaaaagtgggaccgagtcggtcctttttttt

SEQ ID NO: 38 - DNA, 24 bp, synthetic construct
  source 1..24: mol_type = other DNA
attgtcgtgaagtagagaaacagg

SEQ ID NO: 39 - DNA, 24 bp, synthetic construct
  source 1..24: mol_type = other DNA
aaaccctgtttctctacttcacga

SEQ ID NO: 40 - RNA, 345 nt, synthetic construct
  source 1..345: mol_type = other RNA
gagggcctatttcccatgattccttcatatttgcatatacgatacaaggctgttagagagataattggaattaatttgactgtaaacacaaagatattagtacaaaatacgtgacgtagaaagtaataatttcttgggtagtttgcagttttaaaattatgttttaaaatggactatcatatgcttaccgtaacttgaaagtatttcgatttcttggctttatatatcttgtggaaaggacgagaccgagagagggtctcagttttagtactctgcgaaagcagaatctattaaaacaaggctttatgccgtatttaactccatcctatgggtggggtttttttt

SEQ ID NO: 41 - DNA, 24 bp, synthetic construct
  source 1..24: mol_type = other DNA
caccctgcagcaccaggatcagtg

SEQ ID NO: 42 - DNA, 24 bp, synthetic construct
  source 1..24: mol_type = other DNA
aaaccactgatcctggtgctgcag

SEQ ID NO: 43 - DNA, 54 bp, synthetic construct
  source 1..54: mol_type = other DNA
tcgtcggcagcgtcagatgtgtataagagacagaaactgcttctcctcttggga

SEQ ID NO: 44 - DNA, 57 bp, synthetic construct
  source 1..57: mol_type = other DNA
gtctcgtgggctcggagatgtgtataagagacagcagattccttatctggtgacaca